European Patent Specification EP 3 827 011 B1, published June 19, 2024. Title: Methods and Composition for Targeted Genomic Analysis. Applicant: Ripple Biosolutions LLC Raymond, Christopher K. The sequence listing filed with the application follows.

SEQUENCE LISTING (209 sequences)

SEQ ID NO: 1 - DNA, 10 bp, Artificial sequence
  Synthetic
  misc_feature (1)..(1): C at postiion 1 is phosphorylated
ctcatggaga

SEQ ID NO: 2 - DNA, 10 bp, Artificial sequence
  Synthetic
  misc_feature (1)..(1): A at postiion 1 is phosphorylated
agatgcctct

SEQ ID NO: 3 - DNA, 10 bp, Artificial sequence
  Synthetic
  misc_feature (1)..(1): T at postiion 1 is phosphorylated
tctgcaagag

SEQ ID NO: 4 - DNA, 10 bp, Artificial sequence
  Synthetic
  misc_feature (1)..(1): G at postiion 1 is phosphorylated
gagcattctc

SEQ ID NO: 5 - DNA, 10 bp, Artificial sequence
  Synthetic
  misc_feature (1)..(1): G at postiion 1 is phosphorylated
gataactcgt

SEQ ID NO: 6 - DNA, 10 bp, Artificial sequence
  Synthetic
  misc_feature (1)..(1): C at postiion 1 is phosphorylated
ctgttagacg

SEQ ID NO: 7 - DNA, 10 bp, Artificial sequence
  Synthetic
  misc_feature (1)..(1): A at postiion 1 is phosphorylated
agcggtctac

SEQ ID NO: 8 - DNA, 10 bp, Artificial sequence
  Synthetic
  misc_feature (1)..(1): T at postiion 1 is phosphorylated
tcaccgagta

SEQ ID NO: 9 - DNA, 10 bp, Artificial sequence
  Synthetic
  misc_feature (1)..(1): A at postiion 1 is phosphorylated
accattggtc

SEQ ID NO: 10 - DNA, 10 bp, Artificial sequence
  Synthetic
  misc_feature (1)..(1): C at postiion 1 is phosphorylated
caatggccga

SEQ ID NO: 11 - DNA, 10 bp, Artificial sequence
  Synthetic
  misc_feature (1)..(1): G at postiion 1 is phosphorylated
gttgccaact

SEQ ID NO: 12 - DNA, 10 bp, Artificial sequence
  Synthetic
  misc_feature (1)..(1): T at postiion 1 is phosphorylated
tggcaattag

SEQ ID NO: 13 - DNA, 10 bp, Artificial sequence
  Synthetic
  misc_feature (1)..(1): A at postiion 1 is phosphorylated
actcaagctg

SEQ ID NO: 14 - DNA, 10 bp, Artificial sequence
  Synthetic
  misc_feature (1)..(1): C at postiion 1 is phosphorylated
cagattcagc

SEQ ID NO: 15 - DNA, 10 bp, Artificial sequence
  Synthetic
  misc_feature (1)..(1): G at postiion 1 is phosphorylated
gtctggatca

SEQ ID NO: 16 - DNA, 10 bp, Artificial sequence
  Synthetic
  misc_feature (1)..(1): T at postiion 1 is phosphorylated
tgagcctgat

SEQ ID NO: 17 - DNA, 47 bp, Artificial sequence
  Synthetic
  misc_feature (30)..(37): n is a, c, g, or t
caactccctacacgacgctcttccgatctnnnnnnnntctccatgag

SEQ ID NO: 18 - DNA, 47 bp, Artificial sequence
  Synthetic
  misc_feature (30)..(37): n is a, c, g, or t
caactccctacacgacgctcttccgatctnnnnnnnnagaggcatct

SEQ ID NO: 19 - DNA, 47 bp, Artificial sequence
  Synthetic
  misc_feature (30)..(37): n is a, c, g, or t
caactccctacacgacgctcttccgatctnnnnnnnnctcttgcaga

SEQ ID NO: 20 - DNA, 47 bp, Artificial sequence
  Synthetic
  misc_feature (30)..(37): n is a, c, g, or t
caactccctacacgacgctcttccgatctnnnnnnnngagaatgctc

SEQ ID NO: 21 - DNA, 47 bp, Artificial sequence
  Synthetic
  misc_feature (30)..(37): n is a, c, g, or t
caactccctacacgacgctcttccgatctnnnnnnnnacgagttatc

SEQ ID NO: 22 - DNA, 47 bp, Artificial sequence
  Synthetic
  misc_feature (30)..(37): n is a, c, g, or t
caactccctacacgacgctcttccgatctnnnnnnnncgtctaacag

SEQ ID NO: 23 - DNA, 47 bp, Artificial sequence
  Synthetic
  misc_feature (30)..(37): n is a, c, g, or t
caactccctacacgacgctcttccgatctnnnnnnnngtagaccgct

SEQ ID NO: 24 - DNA, 47 bp, Artificial sequence
  Synthetic
  misc_feature (30)..(37): n is a, c, g, or t
caactccctacacgacgctcttccgatctnnnnnnnntactcggtga

SEQ ID NO: 25 - DNA, 47 bp, Artificial sequence
  Synthetic
  misc_feature (30)..(37): n is a, c, g, or t
caactccctacacgacgctcttccgatctnnnnnnnngaccaatggt

SEQ ID NO: 26 - DNA, 47 bp, Artificial sequence
  Synthetic
  misc_feature (30)..(37): n is a, c, g, or t
caactccctacacgacgctcttccgatctnnnnnnnntcggccattg

SEQ ID NO: 27 - DNA, 47 bp, Artificial sequence
  Synthetic
  misc_feature (30)..(37): n is a, c, g, or t
caactccctacacgacgctcttccgatctnnnnnnnnagttggcaac

SEQ ID NO: 28 - DNA, 47 bp, Artificial sequence
  Synthetic
  misc_feature (30)..(37): n is a, c, g, or t
caactccctacacgacgctcttccgatctnnnnnnnnctaattgcca

SEQ ID NO: 29 - DNA, 47 bp, Artificial sequence
  Synthetic
  misc_feature (30)..(37): n is a, c, g, or t
caactccctacacgacgctcttccgatctnnnnnnnncagcttgagt

SEQ ID NO: 30 - DNA, 47 bp, Artificial sequence
  Synthetic
  misc_feature (30)..(37): n is a, c, g, or t
caactccctacacgacgctcttccgatctnnnnnnnngctgaatctg

SEQ ID NO: 31 - DNA, 47 bp, Artificial sequence
  Synthetic
  misc_feature (30)..(37): n is a, c, g, or t
caactccctacacgacgctcttccgatctnnnnnnnntgatccagac

SEQ ID NO: 32 - DNA, 47 bp, Artificial sequence
  Synthetic
  misc_feature (30)..(37): n is a, c, g, or t
caactccctacacgacgctcttccgatctnnnnnnnnatcaggctca

SEQ ID NO: 33 - DNA, 58 bp, Artificial sequence
  Synthetic
aatgatacggcgaccaccgagatctacactctttccctacacgacgctcttccgatct

SEQ ID NO: 34 - DNA, 21 bp, Artificial sequence
  Synthetic
gaggctgaggcaggagaatcg

SEQ ID NO: 35 - DNA, 58 bp, Artificial sequence; identical to SEQ ID NO: 33
  Synthetic

SEQ ID NO: 36 - DNA, 25 bp, Artificial sequence
  Synthetic
gtcgcagagcacttgcagacttttt

SEQ ID NO: 37 - DNA, 25 bp, Artificial sequence
  Synthetic
aatgtggtttcgttggaagcaaatg

SEQ ID NO: 38 - DNA, 25 bp, Artificial sequence
  Synthetic
ttctgcttaaccattgtgggcatct

SEQ ID NO: 39 - DNA, 25 bp, Artificial sequence
  Synthetic
caatcaagatggttttgccaaggaa

SEQ ID NO: 40 - DNA, 25 bp, Artificial sequence
  Synthetic
cgtatccccctgcatttcttttgtt

SEQ ID NO: 41 - DNA, 25 bp, Artificial sequence
  Synthetic
caaagggtgaagaggaatcccaaag

SEQ ID NO: 42 - DNA, 25 bp, Artificial sequence
  Synthetic
tttatccatcccatcacaccctcag

SEQ ID NO: 43 - DNA, 25 bp, Artificial sequence
  Synthetic
aaagaaaagttctgcatccccagga

SEQ ID NO: 44 - DNA, 83 bp, Artificial sequence
  Synthetic
atacgagatgtgactggagttcagacgtgtgctcttccgatctcccagggttggaagtgtctcatgctggatccccacttttc

SEQ ID NO: 45 - DNA, 83 bp, Artificial sequence
  Synthetic
atacgagatgtgactggagttcagacgtgtgctcttccgatctgaggagccgcagtcagatcctagcgtcgagccccctctga

SEQ ID NO: 46 - DNA, 83 bp, Artificial sequence
  Synthetic
atacgagatgtgactggagttcagacgtgtgctcttccgatcttccactcacagtttccataggtctgaaaatgtttcctgac

SEQ ID NO: 47 - DNA, 83 bp, Artificial sequence
  Synthetic
atacgagatgtgactggagttcagacgtgtgctcttccgatctgaaaattccatgggactgactttctgctcttgtctttcag

SEQ ID NO: 48 - DNA, 83 bp, Artificial sequence
  Synthetic
atacgagatgtgactggagttcagacgtgtgctcttccgatctggctggggggctggggggctgaggacctggtcctctgact

SEQ ID NO: 49 - DNA, 83 bp, Artificial sequence
  Synthetic
atacgagatgtgactggagttcagacgtgtgctcttccgatctcaatggatgatttgatgctgtccccggacgatattgaaca

SEQ ID NO: 50 - DNA, 83 bp, Artificial sequence
  Synthetic
atacgagatgtgactggagttcagacgtgtgctcttccgatctatgccagaggctgctccccccgtggcccctgcaccagcag

SEQ ID NO: 51 - DNA, 83 bp, Artificial sequence
  Synthetic
atacgagatgtgactggagttcagacgtgtgctcttccgatctcctgtcatcttctgtcccttcccagaaaacctaccagggc

SEQ ID NO: 52 - DNA, 83 bp, Artificial sequence
  Synthetic
atacgagatgtgactggagttcagacgtgtgctcttccgatctgcagggggatacggccaggcattgaagtctcatggaagcc

SEQ ID NO: 53 - DNA, 83 bp, Artificial sequence
  Synthetic
atacgagatgtgactggagttcagacgtgtgctcttccgatctctgtcccagaatgcaagaagcccagacggaaaccgtagct

SEQ ID NO: 54 - DNA, 83 bp, Artificial sequence
  Synthetic
atacgagatgtgactggagttcagacgtgtgctcttccgatctggccaggagggggctggtgcaggggccgccggtgtaggag

SEQ ID NO: 55 - DNA, 83 bp, Artificial sequence
  Synthetic
atacgagatgtgactggagttcagacgtgtgctcttccgatcttctgggagcttcatctggacctgggtcttcagtgaaccat

SEQ ID NO: 56 - DNA, 83 bp, Artificial sequence
  Synthetic
atacgagatgtgactggagttcagacgtgtgctcttccgatctttcacttgtgccctgactttcaactctgtctccttcctct

SEQ ID NO: 57 - DNA, 83 bp, Artificial sequence
  Synthetic
atacgagatgtgactggagttcagacgtgtgctcttccgatctactggccaagacctgccctgtgcagctgtgggttgattcc

SEQ ID NO: 58 - DNA, 83 bp, Artificial sequence
  Synthetic
atacgagatgtgactggagttcagacgtgtgctcttccgatctacaagcagtcacagcacatgacggaggttgtgaggcgctg

SEQ ID NO: 59 - DNA, 83 bp, Artificial sequence
  Synthetic
atacgagatgtgactggagttcagacgtgtgctcttccgatctctgctcaccatcgctatctgagcagcgctcatggtggggg

SEQ ID NO: 60 - DNA, 83 bp, Artificial sequence
  Synthetic
atacgagatgtgactggagttcagacgtgtgctcttccgatctagatggccatggcgcggacgcgggtgccgggcgggggtgt

SEQ ID NO: 61 - DNA, 83 bp, Artificial sequence
  Synthetic
atacgagatgtgactggagttcagacgtgtgctcttccgatctagagacgacagggctggttgcccagggtccccaggcctct

SEQ ID NO: 62 - DNA, 83 bp, Artificial sequence
  Synthetic
atacgagatgtgactggagttcagacgtgtgctcttccgatctcatcttatccgagtggaaggaaatttgcgtgtggagtatt

SEQ ID NO: 63 - DNA, 83 bp, Artificial sequence
  Synthetic
atacgagatgtgactggagttcagacgtgtgctcttccgatctcctggagggccactgacaaccacccttaacccctcctccc

SEQ ID NO: 64 - DNA, 83 bp, Artificial sequence
  Synthetic
atacgagatgtgactggagttcagacgtgtgctcttccgatctggcaccaccacactatgtcgaaaagtgtttctgtcatcca

SEQ ID NO: 65 - DNA, 83 bp, Artificial sequence
  Synthetic
atacgagatgtgactggagttcagacgtgtgctcttccgatctcccctgcttgccacaggtctccccaaggcgcactggcctc

SEQ ID NO: 66 - DNA, 83 bp, Artificial sequence
  Synthetic
atacgagatgtgactggagttcagacgtgtgctcttccgatctaccaccatccactacaactacatgtgtaacagttcctgca

SEQ ID NO: 67 - DNA, 83 bp, Artificial sequence
  Synthetic
atacgagatgtgactggagttcagacgtgtgctcttccgatctggtcagaggcaagcagaggctggggcacagcaggccagtg

SEQ ID NO: 68 - DNA, 83 bp, Artificial sequence
  Synthetic
atacgagatgtgactggagttcagacgtgtgctcttccgatctgtgatgatggtgaggatgggcctccggttcatgccgccca

SEQ ID NO: 69 - DNA, 83 bp, Artificial sequence
  Synthetic
atacgagatgtgactggagttcagacgtgtgctcttccgatcttaggacctgatttccttactgcctcttgcttctcttttcc

SEQ ID NO: 70 - DNA, 83 bp, Artificial sequence
  Synthetic
atacgagatgtgactggagttcagacgtgtgctcttccgatctgaggtgcgtgtttgtgcctgtcctgggagagaccggcgca

SEQ ID NO: 71 - DNA, 83 bp, Artificial sequence
  Synthetic
atacgagatgtgactggagttcagacgtgtgctcttccgatctgcataactgcacccttggtctcctccaccgcttcttgtcc

SEQ ID NO: 72 - DNA, 83 bp, Artificial sequence
  Synthetic
atacgagatgtgactggagttcagacgtgtgctcttccgatcttggtgaggctcccctttcttgcggagattctcttcctctg

SEQ ID NO: 73 - DNA, 83 bp, Artificial sequence
  Synthetic
atacgagatgtgactggagttcagacgtgtgctcttccgatctgagaccaagggtgcagttatgcctcagattcacttttatc

SEQ ID NO: 74 - DNA, 83 bp, Artificial sequence
  Synthetic
atacgagatgtgactggagttcagacgtgtgctcttccgatctagctcctctccccagccaaagaagaaaccactggatggag

SEQ ID NO: 75 - DNA, 83 bp, Artificial sequence
  Synthetic
atacgagatgtgactggagttcagacgtgtgctcttccgatcttaagaggtcccaagacttagtacctgaagggtgaaatatt

SEQ ID NO: 76 - DNA, 83 bp, Artificial sequence
  Synthetic
atacgagatgtgactggagttcagacgtgtgctcttccgatctcttgaaccatcttttaactcaggtactgtgtatatactta

SEQ ID NO: 77 - DNA, 83 bp, Artificial sequence
  Synthetic
atacgagatgtgactggagttcagacgtgtgctcttccgatctgcgcttcgagatgttccgagagctgaatgaggccttggaa

SEQ ID NO: 78 - DNA, 83 bp, Artificial sequence
  Synthetic
atacgagatgtgactggagttcagacgtgtgctcttccgatctgaatcctatggctttccaacctaggaaggcaggggagtag

SEQ ID NO: 79 - DNA, 83 bp, Artificial sequence
  Synthetic
atacgagatgtgactggagttcagacgtgtgctcttccgatcttgctcccccctggctccttcccagcctgggcatccttgag

SEQ ID NO: 80 - DNA, 83 bp, Artificial sequence
  Synthetic
atacgagatgtgactggagttcagacgtgtgctcttccgatctggcacagaccctctcactcatgtgatgtcatctctcctcc

SEQ ID NO: 81 - DNA, 83 bp, Artificial sequence
  Synthetic
atacgagatgtgactggagttcagacgtgtgctcttccgatcttcagtctacctcccgccataaaaaactcatgttcaagaca

SEQ ID NO: 82 - DNA, 83 bp, Artificial sequence
  Synthetic
atacgagatgtgactggagttcagacgtgtgctcttccgatctgaacaagaagtggagaatgtcagtctgagtcaggcccttc

SEQ ID NO: 83 - DNA, 83 bp, Artificial sequence
  Synthetic
atacgagatgtgactggagttcagacgtgtgctcttccgatctcaagtgaacagataaagcaactggaagacggcagcaaaga

SEQ ID NO: 84 - DNA, 83 bp, Artificial sequence
  Synthetic
atacgagatgtgactggagttcagacgtgtgctcttccgatcttctgtagctgtagaggcattttaaccctttgtcctccagc

SEQ ID NO: 85 - DNA, 83 bp, Artificial sequence
  Synthetic
atacgagatgtgactggagttcagacgtgtgctcttccgatctcctccctgtctcacgccatggtagcgtccgcctaggttgc

SEQ ID NO: 86 - DNA, 83 bp, Artificial sequence
  Synthetic
atacgagatgtgactggagttcagacgtgtgctcttccgatctcccggttgtccccagatcctgtggctggctcagctgtgtc

SEQ ID NO: 87 - DNA, 83 bp, Artificial sequence
  Synthetic
atacgagatgtgactggagttcagacgtgtgctcttccgatcttcacttgttctatattattattctagagagaactgtgtga

SEQ ID NO: 88 - DNA, 83 bp, Artificial sequence
  Synthetic
atacgagatgtgactggagttcagacgtgtgctcttccgatcttttaaatcccgtaatccttggtgagaggctgccgaggggg

SEQ ID NO: 89 - DNA, 83 bp, Artificial sequence
  Synthetic
atacgagatgtgactggagttcagacgtgtgctcttccgatctgctaagttgcaggtactttttgataactttaggacttggg

SEQ ID NO: 90 - DNA, 83 bp, Artificial sequence
  Synthetic
atacgagatgtgactggagttcagacgtgtgctcttccgatctctccaggcagctggctctggtattcagaatcagaacggac

SEQ ID NO: 91 - DNA, 83 bp, Artificial sequence
  Synthetic
atacgagatgtgactggagttcagacgtgtgctcttccgatctaatcatgtccatcagatgacggcagatgctgtttgcagtc

SEQ ID NO: 92 - DNA, 83 bp, Artificial sequence
  Synthetic
atacgagatgtgactggagttcagacgtgtgctcttccgatcttctccaaaatccactgagcagacaaccacaaacagtgtta

SEQ ID NO: 93 - DNA, 83 bp, Artificial sequence
  Synthetic
atacgagatgtgactggagttcagacgtgtgctcttccgatctaagtgaaaatgtttgacttactggcatgatcagaatgctg

SEQ ID NO: 94 - DNA, 83 bp, Artificial sequence
  Synthetic
atacgagatgtgactggagttcagacgtgtgctcttccgatctaataaagcttctgtcaaactcttagatgaatgactacacc

SEQ ID NO: 95 - DNA, 83 bp, Artificial sequence
  Synthetic
atacgagatgtgactggagttcagacgtgtgctcttccgatcttgttttcatggggctctgagattcttccatcccttctcca

SEQ ID NO: 96 - DNA, 83 bp, Artificial sequence
  Synthetic
atacgagatgtgactggagttcagacgtgtgctcttccgatctggcttttcccatcaacaaggcagagagctgaggattgtct

SEQ ID NO: 97 - DNA, 83 bp, Artificial sequence
  Synthetic
atacgagatgtgactggagttcagacgtgtgctcttccgatcttccacctgaggtagcagtgtgagaggagaggtgattgaga

SEQ ID NO: 98 - DNA, 83 bp, Artificial sequence
  Synthetic
atacgagatgtgactggagttcagacgtgtgctcttccgatctaaactcagaatatacagaatttaaaatattaaagagaaaa

SEQ ID NO: 99 - DNA, 83 bp, Artificial sequence
  Synthetic
atacgagatgtgactggagttcagacgtgtgctcttccgatctagtgtgtggctttcgtacagtcatccctgtacaacctgtt

SEQ ID NO: 100 - DNA, 83 bp, Artificial sequence
  Synthetic
atacgagatgtgactggagttcagacgtgtgctcttccgatctgcatggcctgtaatttctgtgcctcctggaagaatggcca

SEQ ID NO: 101 - DNA, 83 bp, Artificial sequence
  Synthetic
atacgagatgtgactggagttcagacgtgtgctcttccgatcttcctcatggtcttttggttatatctcatttgttccttcct

SEQ ID NO: 102 - DNA, 83 bp, Artificial sequence
  Synthetic
atacgagatgtgactggagttcagacgtgtgctcttccgatctctggctgagaacagggcagtgaaagggaactgggtgacaa

SEQ ID NO: 103 - DNA, 83 bp, Artificial sequence
  Synthetic
atacgagatgtgactggagttcagacgtgtgctcttccgatctcacggaagggtcaggggcaaggactccatgtgatgggtac

SEQ ID NO: 104 - DNA, 83 bp, Artificial sequence
  Synthetic
atacgagatgtgactggagttcagacgtgtgctcttccgatctcgggagctgcagttccccaccccctccatcttgctgcttg

SEQ ID NO: 105 - DNA, 83 bp, Artificial sequence
  Synthetic
atacgagatgtgactggagttcagacgtgtgctcttccgatctaaaacagatgaaaagcaagatacttctagctggccagcca

SEQ ID NO: 106 - DNA, 83 bp, Artificial sequence
  Synthetic
atacgagatgtgactggagttcagacgtgtgctcttccgatctaaccattagtccctgagaaggtggcaggggtgagactaag

SEQ ID NO: 107 - DNA, 83 bp, Artificial sequence
  Synthetic
atacgagatgtgactggagttcagacgtgtgctcttccgatcttaaggctggcttcctaaacttcattctccccaaactgctt

SEQ ID NO: 108 - DNA, 83 bp, Artificial sequence
  Synthetic
atacgagatgtgactggagttcagacgtgtgctcttccgatctctcttgcagcagccagactgccttccgggtcactgccatg

SEQ ID NO: 109 - DNA, 83 bp, Artificial sequence
  Synthetic
atacgagatgtgactggagttcagacgtgtgctcttccgatctggggttggggtgggggtggtgggcctgcccttccaatgga

SEQ ID NO: 110 - DNA, 83 bp, Artificial sequence
  Synthetic
atacgagatgtgactggagttcagacgtgtgctcttccgatcttcagagggggctcgacgctaggatctgactgcggctcctc

SEQ ID NO: 111 - DNA, 83 bp, Artificial sequence
  Synthetic
atacgagatgtgactggagttcagacgtgtgctcttccgatctgctcttttcacccatctacagtcccccttgccgtcccaag

SEQ ID NO: 112 - DNA, 83 bp, Artificial sequence
  Synthetic
atacgagatgtgactggagttcagacgtgtgctcttccgatctatggttcactgaagacccaggtccagatgaagctcccaga

SEQ ID NO: 113 - DNA, 83 bp, Artificial sequence
  Synthetic
atacgagatgtgactggagttcagacgtgtgctcttccgatctctcctacaccggcggcccctgcaccagccccctcctggcc

SEQ ID NO: 114 - DNA, 83 bp, Artificial sequence
  Synthetic
atacgagatgtgactggagttcagacgtgtgctcttccgatctagctacggtttccgtctgggcttcttgcattctgggacag

SEQ ID NO: 115 - DNA, 83 bp, Artificial sequence
  Synthetic
atacgagatgtgactggagttcagacgtgtgctcttccgatctagcccctcagggcaactgaccgtgcaagtcacagacttgg

SEQ ID NO: 116 - DNA, 83 bp, Artificial sequence
  Synthetic
atacgagatgtgactggagttcagacgtgtgctcttccgatctgccctggtaggttttctgggaagggacagaagatgacagg

SEQ ID NO: 117 - DNA, 83 bp, Artificial sequence
  Synthetic
atacgagatgtgactggagttcagacgtgtgctcttccgatctctgctggtgcaggggccacggggggagcagcctctggcat

SEQ ID NO: 118 - DNA, 83 bp, Artificial sequence
  Synthetic
atacgagatgtgactggagttcagacgtgtgctcttccgatcttgttcaatatcgtccggggacagcatcaaatcatccattg

SEQ ID NO: 119 - DNA, 83 bp, Artificial sequence
  Synthetic
atacgagatgtgactggagttcagacgtgtgctcttccgatcttcctacagtactcccctgccctcaacaagatgttttgcca

SEQ ID NO: 120 - DNA, 83 bp, Artificial sequence
  Synthetic
atacgagatgtgactggagttcagacgtgtgctcttccgatctacacccccgcccggcacccgcgtccgcgccatggccatct

SEQ ID NO: 121 - DNA, 83 bp, Artificial sequence
  Synthetic
atacgagatgtgactggagttcagacgtgtgctcttccgatctggaccctgggcaaccagccctgtcgtctctccagccccag

SEQ ID NO: 122 - DNA, 83 bp, Artificial sequence
  Synthetic
atacgagatgtgactggagttcagacgtgtgctcttccgatctcagcgcctcacaacctccgtcatgtgctgtgactgcttgt

SEQ ID NO: 123 - DNA, 83 bp, Artificial sequence
  Synthetic
atacgagatgtgactggagttcagacgtgtgctcttccgatctggaatcaacccacagctgcacagggcaggtcttggccagt

SEQ ID NO: 124 - DNA, 83 bp, Artificial sequence
  Synthetic
atacgagatgtgactggagttcagacgtgtgctcttccgatctgattcctcactgattgctcttaggtctggcccctcctcag

SEQ ID NO: 125 - DNA, 83 bp, Artificial sequence
  Synthetic
atacgagatgtgactggagttcagacgtgtgctcttccgatcttggatgacagaaacacttttcgacatagtgtggtggtgcc

SEQ ID NO: 126 - DNA, 83 bp, Artificial sequence
  Synthetic
atacgagatgtgactggagttcagacgtgtgctcttccgatctagagaccccagttgcaaaccagacctcaggcggctcatag

SEQ ID NO: 127 - DNA, 83 bp, Artificial sequence
  Synthetic
atacgagatgtgactggagttcagacgtgtgctcttccgatctaatactccacacgcaaatttccttccactcggataagatg

SEQ ID NO: 128 - DNA, 83 bp, Artificial sequence
  Synthetic
atacgagatgtgactggagttcagacgtgtgctcttccgatctatcttgggcctgtgttatctcctaggttggctctgactgt

SEQ ID NO: 129 - DNA, 83 bp, Artificial sequence
  Synthetic
atacgagatgtgactggagttcagacgtgtgctcttccgatcttgggcggcatgaaccggaggcccatcctcaccatcatcac

SEQ ID NO: 130 - DNA, 83 bp, Artificial sequence
  Synthetic
atacgagatgtgactggagttcagacgtgtgctcttccgatcttgcagggtggcaagtggctcctgacctggagtcttccagt

SEQ ID NO: 131 - DNA, 83 bp, Artificial sequence
  Synthetic
atacgagatgtgactggagttcagacgtgtgctcttccgatcttgcaggaactgttacacatgtagttgtagtggatggtggt

SEQ ID NO: 132 - DNA, 83 bp, Artificial sequence
  Synthetic
atacgagatgtgactggagttcagacgtgtgctcttccgatcttatcctgagtagtggtaatctactgggacggaacagcttt

SEQ ID NO: 133 - DNA, 83 bp, Artificial sequence
  Synthetic
atacgagatgtgactggagttcagacgtgtgctcttccgatcttgcttgcttacctcgcttagtgctccctgggggcagctcg

SEQ ID NO: 134 - DNA, 83 bp, Artificial sequence
  Synthetic
atacgagatgtgactggagttcagacgtgtgctcttccgatcttgcgccggtctctcccaggacaggcacaaacacgcacctc

SEQ ID NO: 135 - DNA, 83 bp, Artificial sequence
  Synthetic
atacgagatgtgactggagttcagacgtgtgctcttccgatctacctttccttgcctctttcctagcactgcccaacaacacc

SEQ ID NO: 136 - DNA, 83 bp, Artificial sequence
  Synthetic
atacgagatgtgactggagttcagacgtgtgctcttccgatctaacggcattttgagtgttagactggaaactttccacttga

SEQ ID NO: 137 - DNA, 83 bp, Artificial sequence
  Synthetic
atacgagatgtgactggagttcagacgtgtgctcttccgatctctccatccagtggtttcttctttggctggggagaggagct

SEQ ID NO: 138 - DNA, 83 bp, Artificial sequence
  Synthetic
atacgagatgtgactggagttcagacgtgtgctcttccgatctcttctccccctcctctgttgctgcagatccgtgggcgtga

SEQ ID NO: 139 - DNA, 83 bp, Artificial sequence
  Synthetic
atacgagatgtgactggagttcagacgtgtgctcttccgatctctcaaggatgcccaggctgggaaggagccaggggggagca

SEQ ID NO: 140 - DNA, 83 bp, Artificial sequence
  Synthetic
atacgagatgtgactggagttcagacgtgtgctcttccgatctggccaggaaggggctgaggtcactcacctggagtgagccc

SEQ ID NO: 141 - DNA, 83 bp, Artificial sequence
  Synthetic
atacgagatgtgactggagttcagacgtgtgctcttccgatctttccaaggcctcattcagctctcggaacatctcgaagcgc

SEQ ID NO: 142 - DNA, 83 bp, Artificial sequence
  Synthetic
atacgagatgtgactggagttcagacgtgtgctcttccgatctctgcttctgtctcctacagccacctgaagtccaaaaaggg

SEQ ID NO: 143 - DNA, 83 bp, Artificial sequence
  Synthetic
atacgagatgtgactggagttcagacgtgtgctcttccgatctgcaggggagggagagatgggggtgggaggctgtcagtggg

SEQ ID NO: 144 - DNA, 83 bp, Artificial sequence
  Synthetic
atacgagatgtgactggagttcagacgtgtgctcttccgatcttgtcttgaacatgagttttttatggcgggaggtagactga

SEQ ID NO: 145 - DNA, 83 bp, Artificial sequence
  Synthetic
atacgagatgtgactggagttcagacgtgtgctcttccgatcttagacgccaactctctctagctcgctagtgggttgcagga

SEQ ID NO: 146 - DNA, 83 bp, Artificial sequence
  Synthetic
atacgagatgtgactggagttcagacgtgtgctcttccgatctggaggctgcagcattaaaaaaagaaaaaggaggttagaga

SEQ ID NO: 147 - DNA, 83 bp, Artificial sequence
  Synthetic
atacgagatgtgactggagttcagacgtgtgctcttccgatcttgatgcaaacctcaatccctccccttctttgaatggtgtg

SEQ ID NO: 148 - DNA, 83 bp, Artificial sequence
  Synthetic
atacgagatgtgactggagttcagacgtgtgctcttccgatctccaaactctgtttccaggggagtggagagagaaactgggt

SEQ ID NO: 149 - DNA, 83 bp, Artificial sequence
  Synthetic
atacgagatgtgactggagttcagacgtgtgctcttccgatctgaggtgtacttgcattaatggagtgggggtgggagcagta

SEQ ID NO: 150 - DNA, 83 bp, Artificial sequence
  Synthetic
atacgagatgtgactggagttcagacgtgtgctcttccgatctcctccggccacggctggcacaaggttctctccctcccctg

SEQ ID NO: 151 - DNA, 83 bp, Artificial sequence
  Synthetic
atacgagatgtgactggagttcagacgtgtgctcttccgatctgcttaatattagatttaaactatttttctttctttttagg

SEQ ID NO: 152 - DNA, 83 bp, Artificial sequence
  Synthetic
atacgagatgtgactggagttcagacgtgtgctcttccgatctcaacaaggcattaccttaaccaaagagagcaagccttcag

SEQ ID NO: 153 - DNA, 83 bp, Artificial sequence
  Synthetic
atacgagatgtgactggagttcagacgtgtgctcttccgatctaataacaatgtgggtactggaacctgtgacaaagtcaata

SEQ ID NO: 154 - DNA, 83 bp, Artificial sequence
  Synthetic
atacgagatgtgactggagttcagacgtgtgctcttccgatctgatctgcttctggttaaccacaaacctagtccacagatca

SEQ ID NO: 155 - DNA, 83 bp, Artificial sequence
  Synthetic
atacgagatgtgactggagttcagacgtgtgctcttccgatctttgcttagatgttgtagtcaaatcagatgtgagaagtatt

SEQ ID NO: 156 - DNA, 83 bp, Artificial sequence
  Synthetic
atacgagatgtgactggagttcagacgtgtgctcttccgatcttgatgaactttcccacactaacctgcatgccttcagaact

SEQ ID NO: 157 - DNA, 83 bp, Artificial sequence
  Synthetic
atacgagatgtgactggagttcagacgtgtgctcttccgatctaggtgttgctgttgaaatggctgaagatggtgaagaggca

SEQ ID NO: 158 - DNA, 83 bp, Artificial sequence
  Synthetic
atacgagatgtgactggagttcagacgtgtgctcttccgatctaggaagtccctcgacactggcagtgctgttaggtgtctct

SEQ ID NO: 159 - DNA, 83 bp, Artificial sequence
  Synthetic
atacgagatgtgactggagttcagacgtgtgctcttccgatctatgctgggaaggcccagtggaagagagaggtcgttcacca

SEQ ID NO: 160 - DNA, 83 bp, Artificial sequence
  Synthetic
atacgagatgtgactggagttcagacgtgtgctcttccgatcttaatcagtatttaacatctttagagaaatttttcttcctt

SEQ ID NO: 161 - DNA, 83 bp, Artificial sequence
  Synthetic
atacgagatgtgactggagttcagacgtgtgctcttccgatctcaatgcaatcatatgcttctgctatgttaagcgtattcaa

SEQ ID NO: 162 - DNA, 83 bp, Artificial sequence
  Synthetic
atacgagatgtgactggagttcagacgtgtgctcttccgatctaggatagagtgaagcgacccatgaacgcattcatcgtgtg

SEQ ID NO: 163 - DNA, 83 bp, Artificial sequence
  Synthetic
atacgagatgtgactggagttcagacgtgtgctcttccgatctgccacacccactctgactcccataaaacccagcggctctg

SEQ ID NO: 164 - DNA, 83 bp, Artificial sequence
  Synthetic
atacgagatgtgactggagttcagacgtgtgctcttccgatctgtctagatttttctagattttgtgtctgttttctccagtt

SEQ ID NO: 165 - DNA, 83 bp, Artificial sequence
  Synthetic
atacgagatgtgactggagttcagacgtgtgctcttccgatctagaaagacaaacaccgcatgatcgcactcatatgtcatat

SEQ ID NO: 166 - DNA, 83 bp, Artificial sequence
  Synthetic
atacgagatgtgactggagttcagacgtgtgctcttccgatctagggctggctctctgactgtgtcctcttcttacctgtccc

SEQ ID NO: 167 - DNA, 83 bp, Artificial sequence
  Synthetic
atacgagatgtgactggagttcagacgtgtgctcttccgatctcaaatggccggagctggaccgaccatgctgctacgagaag

SEQ ID NO: 168 - DNA, 83 bp, Artificial sequence
  Synthetic
atacgagatgtgactggagttcagacgtgtgctcttccgatctgctgtagatcttcttcgattgaccactgtgatggaaactg

SEQ ID NO: 169 - DNA, 83 bp, Artificial sequence
  Synthetic
atacgagatgtgactggagttcagacgtgtgctcttccgatctagattatcatatgagaactcccttgaaattccaatactca

SEQ ID NO: 170 - DNA, 83 bp, Artificial sequence
  Synthetic
atacgagatgtgactggagttcagacgtgtgctcttccgatcttgctggggccatcacgatgtgtgggtgtccaggcctccgg

SEQ ID NO: 171 - DNA, 43 bp, Artificial sequence
  Synthetic
agatcggaagagcacacgtctgaactccagtcacauctcguat

SEQ ID NO: 172 - DNA, 41 bp, Artificial sequence
  Synthetic
aatgatacggcgaccaccgagatctacactctttccctaca

SEQ ID NO: 173 - DNA, 44 bp, Artificial sequence
  Synthetic
caagcagaagacggcatacgagatgtgactggagttcagacgtg

SEQ ID NO: 174 - DNA, 21 bp, Homo sapiens
aggggccacgcggggagcagc

SEQ ID NO: 175 - DNA, 21 bp, Homo sapiens
aggggccacggggggagcagc

SEQ ID NO: 176 - DNA, 21 bp, Homo sapiens
aacatattgacggtgcctgaa

SEQ ID NO: 177 - DNA, 20 bp, Homo sapiens
aacatattgaaggtgcctga

SEQ ID NO: 178 - DNA, 21 bp, Homo sapiens
aggtgcttacacatgtttgtt

SEQ ID NO: 179 - DNA, 21 bp, Homo sapiens
aggtgcttacgcatgtttgtt

SEQ ID NO: 180 - DNA, 21 bp, Homo sapiens
atcccttcacttcctcatcct

SEQ ID NO: 181 - DNA, 21 bp, Homo sapiens
atcccttcacgtcctcatcct

SEQ ID NO: 182 - DNA, 21 bp, Homo sapiens
tccccctcccgtagctcctgg

SEQ ID NO: 183 - DNA, 21 bp, Homo sapiens
tccccctcccctagctcctgg

SEQ ID NO: 184 - DNA, 21 bp, Homo sapiens
ttgttagtgcggatctgtggt

SEQ ID NO: 185 - DNA, 21 bp, Homo sapiens
ttgttagtgcagatctgtggt

SEQ ID NO: 186 - DNA, 21 bp, Homo sapiens
gcttctaggactgggctgctt

SEQ ID NO: 187 - DNA, 21 bp, Homo sapiens
gcttctaggattgggctgctt

SEQ ID NO: 188 - DNA, 21 bp, Homo sapiens
tactaagtcttgggacctctt

SEQ ID NO: 189 - DNA, 21 bp, Homo sapiens
tactaagtctcgggacctctt

SEQ ID NO: 190 - DNA, 21 bp, Homo sapiens
gggttggggtcggggtggtgg

SEQ ID NO: 191 - DNA, 21 bp, Homo sapiens
gggttggggtgggggtggtgg

SEQ ID NO: 192 - DNA, 21 bp, Homo sapiens
taagaggtgggcccaggggtc

SEQ ID NO: 193 - DNA, 21 bp, Homo sapiens
taagaggtggacccaggggtc

SEQ ID NO: 194 - DNA, 21 bp, Homo sapiens
ccagttttactccaatctcct

SEQ ID NO: 195 - DNA, 21 bp, Homo sapiens
ccagttttaccccaatctcct

SEQ ID NO: 196 - DNA, 21 bp, Homo sapiens
cagttgatccgacagcaacag

SEQ ID NO: 197 - DNA, 21 bp, Homo sapiens
cagttgatccaacagcaacag

SEQ ID NO: 198 - DNA, 21 bp, Homo sapiens
gtaaccagcactcgactctgc

SEQ ID NO: 199 - DNA, 21 bp, Homo sapiens
gtaaccagcaatcgactctgc

SEQ ID NO: 200 - DNA, 21 bp, Homo sapiens
ggcagcgactcagcctgtcct

SEQ ID NO: 201 - DNA, 21 bp, Homo sapiens
ggcagcgacttagcctgtcct

SEQ ID NO: 202 - DNA, 21 bp, Homo sapiens
tgctaaccccagcactggagc

SEQ ID NO: 203 - DNA, 21 bp, Homo sapiens
tgctaaccccggcactggagc

SEQ ID NO: 204 - DNA, 21 bp, Homo sapiens
caatgtcaaatgggaaaaagt

SEQ ID NO: 205 - DNA, 21 bp, Homo sapiens
caatgtcaaacgggaaaaagt

SEQ ID NO: 206 - DNA, 21 bp, Homo sapiens
gacaggaggacaggataaaag

SEQ ID NO: 207 - DNA, 21 bp, Homo sapiens
gacaggaggaaaggataaaag

SEQ ID NO: 208 - DNA, 21 bp, Homo sapiens
ggacctagatgccaggaccat

SEQ ID NO: 209 - DNA, 21 bp, Homo sapiens
ggacctagattccaggaccat